European Patent Specification EP 3 791 889 B1, published February 21, 2024. Title: RECEPTOR TARGETING CONSTRUCTS AND USES THEREOF. Applicant: CEDARS-SINAI MEDICAL CENTER. The sequence listing filed with the application follows.

SEQUENCE LISTING (13 sequences)

SEQ ID NO: 1 - DNA, 24 bp, Homo sapiens
agtgagctcgagactatcactgtg

SEQ ID NO: 2 - DNA, 51 bp, Homo sapiens
gttggtgactttctcccaccttcaccaccttcatctagatatccatggtat

SEQ ID NO: 3 - protein, 6 aa, Artificial Sequence
  Synthesized sequence
GGSGGS

SEQ ID NO: 4 - DNA, 30 bp, Homo sapiens
cgcctgagcaacgcggcgggcatccgcaag

SEQ ID NO: 5 - protein, 44 aa, Human immunodeficiency virus
TITLPCRIKQFINMWQEVGKAMYAPPISGQIRCSSNITGLLLTR

SEQ ID NO: 6 - DNA, 30 bp, Yersinia enterocolitica
acagagctcataaccggcattaacgtgaat

SEQ ID NO: 7 - DNA, 30 bp, Yersinia enterocolitica
ctgtgtgcggagccgcaataggaattcatc

SEQ ID NO: 8 - DNA, 30 bp, Yersinia enterocolitica
gatgaattcctattgcggctccgcacacag

SEQ ID NO: 9 - DNA, 33 bp, Yersinia enterocolitica
gtccaaaaccaagaaaaggcggagcagctgtac

SEQ ID NO: 10 - DNA, 45 bp, Yersinia enterocolitica
acaatgacgcgtgtacagctgctccgccttttcttggttttggac

SEQ ID NO: 11 - DNA, 39 bp, Yersinia enterocolitica
ccgctgtgtgcggagccgcaaggaggaacgcgtacacac

SEQ ID NO: 12 - DNA, 39 bp, Yersinia enterocolitica
gtgtgtacgcgttcctccttgcggctccgcacacagcgg

SEQ ID NO: 13 - DNA, 33 bp, Yersinia enterocolitica
acacacggatccttgcggctccgcacacagcgg